European Patent Specification EP 4 185 707 B1, published August 28, 2024. Title: BASE-MODIFIED NUCLEOTIDES AS SUBSTRATES FOR TDT-BASED ENZYMATIC NUCLEIC ACID SYNTHESIS. Applicant: Illumina Singapore Pte. Ltd. Nanyang Technological University Ee, Pin Koon Teo, Yin Nah Chiba, Shunsuke. The sequence listing filed with the application follows.

SEQUENCE LISTING (1 sequence)

SEQ ID NO: 1 - DNA, 21 bp, Artificial Sequence
  Synthetic Oligonucleotide
attcaggacgagcctcagacc